European Patent Application EP 4 276 171 A1, published November 15, 2023. Title: BACILLUS SUBTILIS GENETICALLY ENGINEERED BACTERIUM FOR PRODUCING TAGATOSE AND METHOD FOR PREPARING TAGATOSE. Applicant: TIANJIN INSTITUTE OF INDUSTRIAL BIOTECHNOLOGY, CHINESE ACADEMY OF SCIENCES. The sequence listing filed with the application follows.

SEQUENCE LISTING (32 sequences)

SEQ ID NO: 1 - DNA, 50 bp, Artificial Sequence
agaaacaacaaagggggagatttgtatggtgaacgtttccaatgccgttg

SEQ ID NO: 2 - DNA, 51 bp, Artificial Sequence
gcttgagctcgactctagaggatcctcagtcaagtcccttccacttgacca

SEQ ID NO: 3 - DNA, 51 bp, Artificial Sequence
tggtcaagtggaagggacttgactgaggatcctctagagtcgagctcaagc

SEQ ID NO: 4 - DNA, 50 bp, Artificial Sequence
caacggcattggaaacgttcaccatacaaatctccccctttgttgtttct

SEQ ID NO: 5 - DNA, 50 bp, Artificial Sequence
agaaacaacaaagggggagatttgtatgggcaaactgtttggtaccttcg

SEQ ID NO: 6 - DNA, 51 bp, Artificial Sequence
agcttgagctcgactctagaggatccttaacctttcagtgcttcttccagc

SEQ ID NO: 7 - DNA, 51 bp, Artificial Sequence
gctggaagaagcactgaaaggttaaggatcctctagagtcgagctcaagct

SEQ ID NO: 8 - DNA, 50 bp, Artificial Sequence
cgaaggtaccaaacagtttgcccatacaaatctccccctttgttgtttct

SEQ ID NO: 9 - DNA, 50 bp, Artificial Sequence
agaaacaacaaagggggagatttgtatgctgcgtctggatactcgctttc

SEQ ID NO: 10 - DNA, 51 bp, Artificial Sequence
agcttgagctcgactctagaggatccttaaccagccaggcgtttacgagtc

SEQ ID NO: 11 - DNA, 51 bp, Artificial Sequence
gactcgtaaacgcctggctggttaaggatcctctagagtcgagctcaagct

SEQ ID NO: 12 - DNA, 50 bp, Artificial Sequence
agaaacaacaaagggggagatttgtatgaaagtttggctggttggtgcct

SEQ ID NO: 13 - DNA, 51 bp, Artificial Sequence
agcttgagctcgactctagaggatccttatttcaggttgctataccattct

SEQ ID NO: 14 - DNA, 51 bp, Artificial Sequence
agaatggtatagcaacctgaaataaggatcctctagagtcgagctcaagct

SEQ ID NO: 15 - DNA, 50 bp, Artificial Sequence
aggcaccaaccagccaaactttcatacaaatctccccctttgttgtttct

SEQ ID NO: 16 - DNA, 50 bp, Artificial Sequence
gaaagcgagtatccagacgcagcatacaaatctccccctttgttgtttct

SEQ ID NO: 17 - DNA, 50 bp, Artificial Sequence
agaaacaacaaagggggagatttgtatgttcaagccgaaagcgatcgcgg

SEQ ID NO: 18 - DNA, 50 bp, Artificial Sequence
agcttgagctcgactctagaggatccttaacgcagcaggcccagaaactg

SEQ ID NO: 19 - DNA, 50 bp, Artificial Sequence
cagtttctgggcctgctgcgttaaggatcctctagagtcgagctcaagct

SEQ ID NO: 20 - DNA, 50 bp, Artificial Sequence
ccgcgatcgctttcggcttgaacatacaaatctccccctttgttgtttct

SEQ ID NO: 21 - DNA, 50 bp, Artificial Sequence; identical to SEQ ID NO: 1

SEQ ID NO: 22 - DNA, 66 bp, Artificial Sequence
cgaaggtaccaaacagtttgcccattttgaattcctccttttcagtcaagtcccttccacttgacc

SEQ ID NO: 23 - DNA, 66 bp, Artificial Sequence
ggtcaagtggaagggacttgactgaaaaggaggaattcaaaatgggcaaactgtttggtaccttcg

SEQ ID NO: 24 - DNA, 66 bp, Artificial Sequence
gaaagcgagtatccagacgcagcattttgaattcctcctttttaacctttcagtgcttcttccagc

SEQ ID NO: 25 - DNA, 66 bp, Artificial Sequence
gctggaagaagcactgaaaggttaaaaaggaggaattcaaaatgctgcgtctggatactcgctttc

SEQ ID NO: 26 - DNA, 66 bp, Artificial Sequence
ttttcagcggatgttcggtgttcattttgaattcctccttttcaaccagccaggcgtttacgagtc

SEQ ID NO: 27 - DNA, 66 bp, Artificial Sequence
gactcgtaaacgcctggctggttgaaaaggaggaattcaaaatgaacaccgaacatccgctgaaaa

SEQ ID NO: 28 - DNA, 67 bp, Artificial Sequence
accgcgatcgctttcggcttgaacattttgaattcctcctttttaaatcagtttgaattcaccgctg

SEQ ID NO: 29 - DNA, 67 bp, Artificial Sequence
cagcggtgaattcaaactgatttaaaaaggaggaattcaaaatgttcaagccgaaagcgatcgcggt

SEQ ID NO: 30 - DNA, 51 bp, Artificial Sequence
gcttgagctcgactctagaggatccttaacgcagcaggcccagaaactgca

SEQ ID NO: 31 - DNA, 51 bp, Artificial Sequence
tgcagtttctgggcctgctgcgttaaggatcctctagagtcgagctcaagc

SEQ ID NO: 32 - DNA, 50 bp, Artificial Sequence; identical to SEQ ID NO: 4